European Patent Application EP 4 772 652 A1, published July 8, 2026. Title: 식물 캘러스 유래 엑소좀 검증용 바이오마커. Applicant: (주)지에프씨생명과학. The sequence listing filed with the application follows.

SEQUENCE LISTING (48 sequences)

SEQ ID NO: 1 - RNA, 21 nt, Leontopodium alpinum
  source 1..21: mol_type = other RNA
ugacagaagagagugagcacc

SEQ ID NO: 2 - RNA, 21 nt, Centella asiatica
  source 1..21: mol_type = other RNA
ugacagaagagagugagcaca

SEQ ID NO: 3 - RNA, 21 nt, Leontopodium alpinum
  source 1..21: mol_type = other RNA
uugacagaagauagagagcac

SEQ ID NO: 4 - RNA, 20 nt, Leontopodium alpinum
  source 1..20: mol_type = other RNA
uuggacugaagggagcuccc

SEQ ID NO: 5 - RNA, 20 nt, Leontopodium alpinum
  source 1..20: mol_type = other RNA
cucaacuucaagcaaagcuu

SEQ ID NO: 6 - RNA, 21 nt, Leontopodium alpinum
  source 1..21: mol_type = other RNA
ucggaccaggcuucauucccc

SEQ ID NO: 7 - RNA, 21 nt, Centella asiatica
  source 1..21: mol_type = other RNA
ucaggucaucuugcagcuuca

SEQ ID NO: 8 - RNA, 21 nt, Centella asiatica
  source 1..21: mol_type = other RNA
ucgcuuggugcaggucgggac

SEQ ID NO: 9 - RNA, 22 nt, Leontopodium alpinum
  source 1..22: mol_type = other RNA
uguaauccuuagcuuugugguu

SEQ ID NO: 10 - RNA, 21 nt, Leontopodium alpinum
  source 1..21: mol_type = other RNA
ugauugagccgugccaauauc

SEQ ID NO: 11 - RNA, 20 nt, Centella asiatica
  source 1..20: mol_type = other RNA
agaugauuuauauguuacug

SEQ ID NO: 12 - RNA, 21 nt, Leontopodium alpinum
  source 1..21: mol_type = other RNA
gcugcuuuacaaugucucuau

SEQ ID NO: 13 - RNA, 21 nt, Centella asiatica
  source 1..21: mol_type = other RNA
uccaaagggaucgcauugauc

SEQ ID NO: 14 - RNA, 20 nt, Centella asiatica
  source 1..20: mol_type = other RNA
cugaaguguuugggggaacu

SEQ ID NO: 15 - RNA, 20 nt, Leontopodium alpinum
  source 1..20: mol_type = other RNA
uuccacagcuuucuugaacu

SEQ ID NO: 16 - RNA, 21 nt, Leontopodium alpinum
  source 1..21: mol_type = other RNA
ucauugagugcagcguugaug

SEQ ID NO: 17 - RNA, 21 nt, Leontopodium alpinum
  source 1..21: mol_type = other RNA
cauguguucucaugucacacc

SEQ ID NO: 18 - RNA, 20 nt, Leontopodium alpinum
  source 1..20: mol_type = other RNA
uuccacagcuuucuugaacu

SEQ ID NO: 19 - RNA, 21 nt, Leontopodium alpinum
  source 1..21: mol_type = other RNA
aucucccucaaaggcuuccaa

SEQ ID NO: 20 - RNA, 21 nt, Centella asiatica
  source 1..21: mol_type = other RNA
gguguggcgucucuggggagg

SEQ ID NO: 21 - RNA, 22 nt, Centella asiatica
  source 1..22: mol_type = other RNA
uuuccuauuccacccaucccau

SEQ ID NO: 22 - RNA, 21 nt, Centella asiatica
  source 1..21: mol_type = other RNA
uuagaugaccaucaacaaacu

SEQ ID NO: 23 - RNA, 22 nt, Leontopodium alpinum
  source 1..22: mol_type = other RNA
ucagaguuuugccaguuccgcc

SEQ ID NO: 24 - RNA, 20 nt, Leontopodium alpinum
  source 1..20: mol_type = other RNA
aaccaggcucugauaccaug

SEQ ID NO: 25 - RNA, 22 nt, Centella asiatica
  source 1..22: mol_type = other RNA
ucauuuuugcgugcaaugaucc

SEQ ID NO: 26 - RNA, 22 nt, Leontopodium alpinum
  source 1..22: mol_type = other RNA
uaaacagugcccacccuucauc

SEQ ID NO: 27 - RNA, 22 nt, Leontopodium alpinum
  source 1..22: mol_type = other RNA
cagaggaagcagcacuuguacc

SEQ ID NO: 28 - RNA, 21 nt, Leontopodium alpinum
  source 1..21: mol_type = other RNA
aaguugugaugagaaucaaug

SEQ ID NO: 29 - RNA, 22 nt, Leontopodium alpinum
  source 1..22: mol_type = other RNA
uuuuagcaagaguuguuuuacc

SEQ ID NO: 30 - RNA, 18 nt, Leontopodium alpinum
  source 1..18: mol_type = other RNA
gucguuguaguauagugg

SEQ ID NO: 31 - RNA, 22 nt, Leontopodium alpinum
  source 1..22: mol_type = other RNA
aacaggaauuucggcucugaua

SEQ ID NO: 32 - RNA, 21 nt, Leontopodium alpinum
  source 1..21: mol_type = other RNA
agggagcucccuucaguccaa

SEQ ID NO: 33 - RNA, 21 nt, Leontopodium alpinum
  source 1..21: mol_type = other RNA
guugaagagucauuguggccc

SEQ ID NO: 34 - RNA, 20 nt, Leontopodium alpinum
  source 1..20: mol_type = other RNA
ucgguuuugauuauucuacu

SEQ ID NO: 35 - RNA, 21 nt, Leontopodium alpinum
  source 1..21: mol_type = other RNA
ucuauggguuuguugauugcc

SEQ ID NO: 36 - RNA, 21 nt, Centella asiatica
  source 1..21: mol_type = other RNA
gguguggcgucucuggggagg

SEQ ID NO: 37 - RNA, 22 nt, Centella asiatica
  source 1..22: mol_type = other RNA
uuggucgguggucuaugucaca

SEQ ID NO: 38 - RNA, 21 nt, Centella asiatica
  source 1..21: mol_type = other RNA
ucugaaagauuguuugugggg

SEQ ID NO: 39 - RNA, 20 nt, Centella asiatica
  source 1..20: mol_type = other RNA
uagaaaacucauaaucgacu

SEQ ID NO: 40 - RNA, 20 nt, Panax ginseng
  source 1..20: mol_type = other RNA
cugcgucgcuccgauucguc

SEQ ID NO: 41 - DNA, 23 bp, synthetic construct
  source 1..23: mol_type = other DNA
gctgaaggaacttctggaaaagg

SEQ ID NO: 42 - DNA, 24 bp, synthetic construct
  source 1..24: mol_type = other DNA
gttgtggtctatatccaagtgatc

SEQ ID NO: 43 - DNA, 22 bp, synthetic construct
  source 1..22: mol_type = other DNA
gccttgctcttcctcatcgttc

SEQ ID NO: 44 - RNA, 22 nt, synthetic construct
  source 1..22: mol_type = other RNA
tgcttgccactggtcaggtaga

SEQ ID NO: 45 - DNA, 22 bp, synthetic construct
  source 1..22: mol_type = other DNA
gattccctggacctaaaggtgc

SEQ ID NO: 46 - DNA, 22 bp, synthetic construct
  source 1..22: mol_type = other DNA
agcctctccatctttgccagca

SEQ ID NO: 47 - DNA, 22 bp, synthetic construct
  source 1..22: mol_type = other DNA
caccattggcaatgagcggttc

SEQ ID NO: 48 - DNA, 22 bp, synthetic construct
  source 1..22: mol_type = other DNA
aggtctttgcggatgtccacgt